European Patent Specification EP 3 077 820 B1, published February 26, 2025. Title: PROTEINS AND NUCLEIC ACIDS USEFUL IN VACCINES TARGETING STAPHYLOCOCCUS AUREUS. Applicant: Novvac ApS. The sequence listing filed with the application follows.

SEQUENCE LISTING (51 sequences)

SEQ ID NO: 1 - protein, 140 aa, Staphylococcus aureus
MAKGNLFKAILGIGGAVAAVLVTRKDSRDKLKAEYNKYKQDPQSYKDNAKDKATQLGTIANETIKEVKTNPKEYANRLKNNPKAFFEEEKSKFTEYDNKTDESIEKGKFDDEGGAAPNNNLRIVTEEDLKKNKNALSDKE

SEQ ID NO: 2 - protein, 193 aa, Staphylococcus aureus
MKKLVSIVGATLLLAGCGSQNLAPLEEKTTDLREDNHQLKLDIQELNQQISDSKSKIKGLEKDKENSKKTASNNTKIKLMNVTSTYYDKVAKALKSYNDIEKDVSKNKGDKNVQSKLNQISNDIQSAHTSYKDAIDGLSLSDDDKKTSKNIDKLNSDLNHAFDDIKNGYQNKDKKQLTKGQQALSKLNLNAKS

SEQ ID NO: 3 - protein, 209 aa, Staphylococcus aureus
MKKLVTGLLALSLFLAACGQDSDQQKDSNKEKDDKAKTEQQDKKTNDSSKDKKDNKDDSKDVNKDNKDNSANDNQQQSNSNATNNDQNQTNNNQSNSGQTTNNQKSSYVAPYYGQNAAPVARQIYPFNGNKSQALQQLPNFQTALNAANNEANKFGNGHKVYNDYSIEEHNGNYKYVFSFKDPNVNGKYSIVTVDYTGQAMVTDPNYQQ

SEQ ID NO: 4 - protein, 242 aa, Staphylococcus aureus
MKKVMGILLASTLILGACGHHQDSAKKESTSHKKKENDNEELNEELKEFKSKKNMDIKIKGDTIVSDKFEAKIKEPFIINEKDEKKKYIAFKMEITAKKDDKDLNPSSISHDYINITQDDKNTVNKLRDGYLLSDKNYKDWTEHNQDQIKKGKTAQAMFIYELRGDGNINLNVHKYSEDKTVDSKSFKFSKLKTEDFSHRAETREEVEKKEKEFEEEYKKEQEREKEKEKQKDDDHSGLDEV

SEQ ID NO: 5 - protein, 327 aa, Staphylococcus aureus
MKKWQFVGTTALGATLLLGACGGGNGGSGNSDLKGEAKGDGSSTVAPIVEKLNEKWAQDHSDAKISAGQAGTGAGFQKFIAGDIDFADASRPIKDEEKQKLQDKNIKYKEFKIAQDGVTVAVNKENDFVDELDKQQLKAIYSGKAKTWKDVNSKWPDKKINAVSPNSSHGTYDFFENEVMNKEDIKAEKNADTNAIVSSVTKNKEGIGYFGYNFYVQNKDKLKEVKIKDENGKATEPTKKTIQDNSYALSRPLFIYVNEKALKDNKVMSEFIKFVLEDKGKAAEEGGYVAAPEKTYKSQLDDLKAFIDKNQKSDDKKSDDKKSEDKK

SEQ ID NO: 6 - protein, 357 aa, Staphylococcus aureus
MKGKFLKVSSLFVATLTTATLVSSPAANALSSKAMDNHPQQTQTDKQQTPKIQKGGNLKPLEQRERANVILPNNDRHQITDTTNGHYAPVTYIQVEAPTGTFIASGVVVGKDTLLTNKHIVDATHGDPHALKAFASAINQDNYPNGGFTAEQITKYSGEGDLAIVKFSPNEQNKHIGEVVKPATMSNNAETQVNQNITVTGYPGDKPVATMWESKGKITYLKGEAMQYDLSTTGGNSGSPVFNEKNEVIGIHWGGVPNQFNGAVFINENVRNFLKQNIEDINFANDDHPNNPDNPDNPNNPDNPNNPDNPNNPDNPDNPNNPDNPNNPDNPNNPDQPNNPNNPDNGDNNNSDNPDAA

SEQ ID NO: 7 - protein, 399 aa, Staphylococcus aureus
MKRTLVLLITAIFILAACGNHKDDQAGKDNQKHNNSSNQVKEIATDKNVQGDNYRTLLPFKESQARGLLQDNMANSYNGGDFEDGLLNLSKEVFPTDKYLYQDGQFLDKKTINAYLNLKYTKREIDKMSEKDKKDKKANENLGLNPSHEGETDPEKIAEKSPAYLSNILEQDFYGGGDTKGKNIKGMTIGLAMNSVYYYKKEKDGPTFSKKLDDSEVKKQGKQMASEILSRLRENDDLKDIPIHFAIYKQSSEDSITPGEFITQATAEKSQTKLNEWHNINEKSALLPSSTAADYDENLNNNFKQFNDNLQSYFSNFTQAVGKVKFVDKKPQRLVVDLPIDYYGQAETIGITQYVTEQANKYFDKIDNYEIRIKDGNQPRALISKTKDDKEPQVHIYSN

SEQ ID NO: 8 - protein, 495 aa, Staphylococcus aureus
MRENFKLRKMKVGLVSVAITMLYIMTNGQAEASEANEKPSTNQESKVVSQTEQNSKETKTVESNKNFVKLDTIKPGAQKITGTTLPNHYVLLTVDGKSADSVENGGLGFVEANDKGEFEYPLNNRKIVHNQEIEVSSSSPDLGEDEEDEEVEEASTDKAGVEEESTEAKVTYTTPRYEKAYEIPKEQLKEKDGHHQVFIEPITEGSGIIKGHTSVKGKVALSINNKFINFEESVKGGVSKEDTKASSDGIWMPIDDKGYFNFDFKTKRFDNLELKEGNDISLTFAPDDEEDALKPLIFKTKVTSLEDIDKAETKYDHTKLNKVKVLDNVKEDLHVDEIYGSLYHTDKGKGILDKEGTKVIKGKTKFANAVVKVDSELGEAQLFPDLQVNEKGEFSFDSHGAGFRLQNGEKLNFTVVDPITGDLLSNEFVSKEIDIEETPEQKADREFDEKLENTPAYYKLYGDKIVGFDTNDFPITWFYPLGEKKVERTTPKLEK

SEQ ID NO: 9 - protein, 507 aa, Staphylococcus aureus
MSKKLKIIIPIIIVLLLIGGIAWGVYAFFANTPKNTYLKSEQQTAKMYKDYFNDRFENEVKFQEKMKDNSFLSSLELSADASDEIVKGLGIPKSVVNASKIKMSYGHDPKKEKSMINLEPTIADSALGKFQLAADKDKHYFESPLFKGKYSVNNSDLLSTYSKLTGEDEETAKENGITNQQLNLNTLFSNAQAQQSDYSKIAEKYSELIVDKLDDDNFDKGKKEEIKVNGEKYKVRPVTLTLSRADTKKITLAVLEEAKKDKDLKKLMEEQGTTKDFEKDIKKAIDDVKETKKDEFAKIQSKIYTEKHTIVKREITITDKENNKTKIKGTNTLEDDKLKLDYALDFDQDKYTYAEAKYTIKGVSSKEKDNKYSDKYEFGKKTEYDESKIKLDNQEKVDGTKRQDKGKITVALDKYSDENEFTFENNIDSDVKNNTQKSTLNIGIKYAEEPINFILKSSTKLKADIDFDDSGAKDFNSLSSKDREKLEKEIEKNGGKMFESILKKASK

SEQ ID NO: 10 - protein, 509 aa, Staphylococcus aureus
MRKFSRYAFTSMATVTLLSSLTPAALASDTNHKPATSDINFEITQKSDAVKALKELPKSENVKNHYQDYSVTDVKTDKKGFTHYTLQPSVDGVHAPDKEVKVHADKSGKVVLINGDTDAKKVKPTNKVTLSKDEAADKAFNAVKIDKNKAKNLQDDVIKENKVEIDGDSNKYIYNIELITVTPEISHWKVKIDADTGAVVEKTNLVKEAAATGTGKGVLGDTKDININSIDGGFSLEDLTHQGKLSAYNFNDQTGQATLITNEDENFVKDDQRAGVDANYYAKQTYDYYKNTFGRESYDNHGSPIVSLTHVNHYGGQDNRNNAAWIGDKMIYGDGDGRTFTNLSGANDVVAHELTHGVTQETANLEYKDQSGALNESFSDVFGYFVDDEDFLMGEDVYTPGKEGDALRSMSNPEQFGQPSHMKDYVYTEKDNGGVHTNSGIPNKAAYNVIQAIGKSKSEQIYYRALTEYLTSNSNFKDCKDALYQAAKDLYDEQTAEQVYEAWNEVGVE

SEQ ID NO: 11 - protein, 515 aa, Staphylococcus aureus
MKKKLGMLLLVPAVTLSLAACGNDDGKDKDGKVTIKTTVYPLQSFAEQIGGKHVKVSSIYPAGTDLHSYEPTQKDILSASKSDLFMYTGDNLDPVAKKVASTIKDKDKKLSLEDKLDKAKLLTDQHEHGEEHEHEGHDHGKEEHHHHGGYDPHVWLDPKINQTFAKEIKDELVKKDPKHKDDYEKNYKKLNDDLKKIDNDMKQVTKDKQGNAVFISHESIGYLADRYGFVQKGIQNMNAEDPSQKELTKIVKEIRDSNAKYILYEDNVANKVTETIRKETDAKPLKFYNMESLNKEQQKKDNITYQSLMKSNIENIGKALDSGVKVKDDKAESKHDKAISDGYFKDEQVKDRELSDYAGEWQSVYPYLKDGTLDEVMEHKAENDPKKSAKDLKAYYDKGYKTDITNIDIKGNEITFTKDGTKHTGKYEYNGKKTLKYPKGNRGVRFMFKLVDGNDKDLPKFIQFSDHNIAPKKAEHFHIFMGNDNDALLKEMDNWPTYYPSKLNKDQIKEEMLAH

SEQ ID NO: 12 - protein, 564 aa, Staphylococcus aureus
MVLYIILAIIVIILIAVGVLFYLRSNKRQIIEKAIERKNEIETLPFDQNLAQLSKLNLKGETKTKYDAMKKDNVESTNKYLAPVEEKIHNAEALLDKFSFNASQCEIDDANELMDSYEQSYQQQLEDVNEIIALYKDNDELYDKCKVDYREMKRDVLANRHQFGEAASLLETEIEKFEPRLEQYEVLKADGNYVQAHNHIAALNEQMKQLRSYMEEIPELIRETQKELPGQFQDLKYGCRDLKVEGYDLDHVKVDSTLQSLKTELSFVEPLISRLELEEANDKLANINDKLDDMYDLIEHEVKAKNDVEETKDIITDNLFKAKDMNYTLQTEIEYVRENYYINESDAQSVRQFENEIQSLISVYDDILKEMSKSAVRYSEVQDNLQYLEDHVTVINDKQEKLQNHLIQLREDEAEAEDNLLRVQSKKEEVYRRLLASNLTSVPERFIIMKNEIDHEVRDVNEQFSERPIHVKQLKDKVSKIVIQMNTFEDEANDVLVNAVYAEKLIQYGNRYRKDYSNVDKSLNEAERLFKNNRYKRAIEIAEQALESVEPGVTKHIEEEVIKQ

SEQ ID NO: 13 - protein, 619 aa, Staphylococcus aureus
MPKNKILIYLLSTTLVLPTLVSPTAYADTPQKDTTAKTTSHDSKKSTDDETSKDTTSKDIDKADNNNTSNQDNNDKKVKTIDDSTSDSNNIIDFIYKNLPQTNINQLLTKNKYDDNYSLTTLIQNLFNLNSDISDYEQPRNGEKSTNDSNKNSDNSIKNDTDTQSSKQDKADNQKAPKSNNTKPSTSNKQPNSPKPTQPNQSNSQPASDDKVNQKSSSKDNQSMSDSALDSILDQYSEDAKKTQKDYASQSKKDKNEKSNTKNPQLPTQDELKHKSKPAQSFNNDVNQKDTRATSLFETDPSISNNDDSGQFNVVDSKDTRQFVKSIAKDAHRIGQDNDIYASVMIAQAILESDSGRSALAKSPNHNLFGIKGAFEGNSVPFNTLEADGNQLYSINAGFRKYPSTKESLKDYSDLIKNGIDGNRTIYKPTWKSEADSYKDATSHLSKTYATDPNYAKKLNSIIKHYQLTQFDDERMPDLDKYERSIKDYDDSSDEFKPFREVSDNMPYPHGQCTWYVYNRMKQFGTSISGDLGDAHNWNNRAQYRDYQVSHTPKRHAAVVFEAGQFGADQHYGHVAFVEKVNSDGSIVISESNVKGLGIISHRTINAAAAEELSYITGK

SEQ ID NO: 14 - protein, 681 aa, Staphylococcus aureus
MMKSQNKYSIRKFSVGASSILIATLLFLSGGQAQAAEKQVNMGNSQEDTVTAQSIGDQQTRENANYQRENGVDEQQHTENLTKNLHNDKTISEENHRKTDDLNKDQLKDDKKSSLNNKNIQRDTTKNNNANPRDVNQGLEQAINDGKQSKVASQQQSKEADNSQDLNANNNLPSQSRTKVSPSLNKSDQTSQREIVNETEIEKVQPQQKNQANDKITDHNFNNEQEVKPQKDEKTLSVSDLKNNQKSPVEPTKDNDKKNGLNLLKSSAVATLPNKGTKELTAKAKGDQTNKVAKQGQYKNQDPIVLVHGFNGFTDDINPSVLAHYWGGNKMNIRQDLEENGYKAYEASISAFGSNYDRAVELYYYIKGGRVDYGAAHAAKYGHERYGKTYEGIYKDWKPGQKVHLVGHSMGGQTIRQLEELLRNGSREEIEYQKKHSGEISPLFKGNNDNMISSITTLGTPHNGTHASDLAGNEALVRQIVFDIGKMFGNKNSRVDFGLAQWGLKQKPNESYIDYVKRVKQSNLWKSKDNGFYDLTREGATDLNRKTSLNPNIVYKTYTGEATHKALNSDRQKADLNMFFPFVITGNLIGKATEKEWRENDGLVSVISSQHPFNQAYTNATDKIQKGIWQVTPTKHDWDHVDFVGQDSSDTVRTREELQDFWHHLADDLVKTEKVTDTKQA

SEQ ID NO: 15 - protein, 806 aa, Staphylococcus aureus
MTNKMKKWQKLSTITLLMTGVIALNNGEFRNVDKHQIAVADTNVQTPDYEKLKKTWLDVNYGYDQYDENNQDMKKKFDAKEKEAKKLLDDMKTDTNRTYLWSGAENLETNSSHMTKTYRNIEKIAESMQHKNTVLKTVENKLKIKEALDWMHKNVYGKNPSQKVEDLTKNRKGQTTPKNNSLNWWDYEIGTPRALTNTLLLMDDMLTKDEMKNYSKPISTYAPSSDKILSSVGESEDAKGGNLVDISKVKLLESVIEEDVDMLKKSIDSFNKVFTYVQDSATGKGRNGFYKDGSYIDHQDVPYTGAYGVVLLEGISQMMPMIKESPFKTTQDNATLSNWIDEGFMPLIYKGEMMDLSRGRAISRENETSHTASATVMKSLLRLNDTMDDSTKTRYKQIVKTSVNSDSSYNQNNYLNSYSDIAKMKKLMNDSTISKNDLTQQLKIYNDMDRVTYHNKDLDFAFGLSMTSKNIARYENINGENLKGWHTGAGMSYLYNSDVKHYRDNFWATADMTCLPGTTTLNDMPSTNTKNDKSFVGGTKLNNKYASIGMDFENQDKTLTAKKSYFILNDKIVFLGTGIKSTDSSKNPVTSVENRKANGYKLFKDDIEITTSDVNAQETHSVFLESNDTKKNIGYHFLDKPKITVKKESHTGKWSEINKSQKKDDKKDEYYEVTQTHNTSDSKYAYVLYPGLSKSDFKSKNNNVSIVKQDEDFHVIKDNDGVFAGVNYSDNTKSFDINGITVELKEKGMFVIKKKDDKAYKCSFYNPETTNTASNIESKIFIKGYTITNKSVINSNDAGVNFELTK

SEQ ID NO: 16 - protein, 808 aa, Staphylococcus aureus
MTYRMKKWQKLSTITLLMAGVITLNGGEFRSIDKHQIAVADTNVQTTDYEKLRNIWLDVNYGYDKYDENNPDMKKKFEATENEAEKLLKEMKTESDRKYLWESSKDLDTKSADMTRTYRNIEKISEAMKHKNTKLKTDENKTKVKDALEWLHKNAYGKEPDKKVADLTSNFKNKTSRNTNLNWWDYEIGTPRALTNTLILLQEDFTDEEKKKYTAPIKTFAPDSDKILSSVGKSEPAKGGNLVDISKVKLLESIIEEDKDMMKKSIDSFNTVFTYAQNSATGKERNGFYKDGSYIDHQDVPYTGAYGVVLLEGISQMMPMIKETPFNDSNQNDTTLKSWIDDGFMPLIYKGEMMDLSRGRAISRENETSHSASATVMKSLLRLSDTMDKSTKAKYKKIVKTSVESDSSYKQTDYLSSYSDISKMKSLMEDSTISTNGLTQQLKIYNDMDRVTYHNKGLDFAFGLSMTSKNVARYESINGENLKGWHTGAGMSYLYNSDVKHYRDNFWATADMKRLAGTTTLDNEEPKSTDVKKSSKTFVGGTKFDDQHASIGMDFENQDKTLTAKKSYFILNDKIVFLGTGIKSTDSSKNPVTTIENRKANDYKLYKDDTQTTNSDNQETNSLFLESTNSTQNNIGYHFLNESKITVKKESHTGKWSDINKSQKDIQKTDEYYEVTQKHSNTDSKYAYVLYPGLSKDVFKSKASKVTVVKQEDDFHVVKDNESVWAGINYSDSAKTFEINNTKVEVKAKGMFILTKKDDNTYECSFYNPESTNSVSDIESKISMTGYSIINKNTSTSNESGVRFELTK

SEQ ID NO: 17 - DNA, 423 bp, Staphylococcus aureus
atggcaaaaggtaatttatttaaagcgattttaggtataggtggcgctgtagcagctgtacttgttacacgtaaagatagtcgtgacaagctgaaagcagaatataataaatacaaacaagatcctcaaagctataaagataatgctaaggataaagcgacgcaattaggaacaattgcaaatgaaacaattaaagaagtaaaaacaaatccgaaagaatatgctaatagattaaaaaataatccaaaagcatttttcgaagaagaaaaatcaaaatttaccgaatatgacaataagactgacgaaagtattgaaaaaggtaaatttgatgatgaaggtggcgcagcaccaaataataatttacgtatcgtcactgaagaagatttaaaaaagaataaaaatgcattgtctgataaagaataa

SEQ ID NO: 18 - DNA, 582 bp, Staphylococcus aureus
atgaaaaaattggtttcaattgttggcgcaacattattgttagctggatgtggatcacaaaatttagcaccattagaagaaaaaacaacagatttaagagaagataatcatcaactcaaactagatattcaagaacttaatcaacaaattagtgattctaaatctaaaattaaagggcttgaaaaggataaagaaaatagtaaaaaaactgcatctaataatacgaaaattaaattgatgaatgttacatcaacatactacgacaaagttgctaaagctttgaaatcctataacgatattgaaaaggatgtaagtaaaaacaaaggcgataagaatgttcaatcgaaattaaatcaaatttctaatgatattcaaagtgctcacacttcatacaaagatgctatcgatggtttatcacttagtgatgatgataaaaaaacgtctaaaaatatcgataaattaaactctgatttgaatcatgcatttgatgatattaaaaatggctatcaaaataaagataaaaaacaacttacaaaaggacaacaagcgttgtcaaaattaaacttaaatgcaaaatcatga

SEQ ID NO: 19 - DNA, 630 bp, Staphylococcus aureus
atgaaaaaattagttacagggttattagcattatcattatttttagctgcatgtggtcaagatagtgaccaacaaaaagacagtaataaagaaaaagatgataaagcgaaaactgaacaacaagataaaaaaacaaatgattcatctaaagataagaaagacaataaagatgatagtaaagacgtaaacaaagataataaagataatagtgcaaacgataaccagcaacaatctaattcaaatgcaacaaacaatgaccaaaatcaaacgaataataaccagtcaaacagtggacaaacgactaacaatcaaaaatcaagttacgttgcaccatattatggacaaaacgcagcgccagtggctcgtcaaatttatccatttaatggtaataaatcacaagcattacaacaattgcctaatttccaaacagctttaaatgcagctaacaacgaagcaaataaatttggtaatggtcataaagtttataatgattattcaattgaagaacataatggtaactataagtatgtttttagttttaaagacccaaacgtaaatggaaaatattcaattgtaacggttgattatactggacaagcaatggttactgatccaaactaccaacaataa

SEQ ID NO: 20 - DNA, 729 bp, Staphylococcus aureus
atgaaaaaagtaatggggatattattagcaagtacacttatcttaggtgcttgtggacatcatcaagatagtgcaaaaaaagagagcactagtcacaaaaagaaagaaaatgacaatgaagaattaaatgaagaacttaaagaatttaaaagcaaaaaaaatatggatataaaaattaaaggcgatactattgttagtgacaaatttgaagctaaaataaaagaaccgtttatcatcaatgaaaaagatgagaaaaagaaatatatcgcttttaaaatggaaattactgctaaaaaagacgataaagatttaaatccatcttctatttctcatgactatattaatatcactcaagatgataaaaatacagtaaataaattaagagatggttatcttttaagtgataaaaattataaagattggacagaacataaccaagatcaaattaaaaaaggcaaaactgcacaagccatgtttatctatgagttaagaggtgatggaaacattaatttaaatgtccataaatactcagaagataaaacagttgattctaaatcattcaaatttagtaaacttaaaaccgaagatttttctcatagagcggaaacaagggaagaagtagaaaagaaagaaaaagaatttgaagaagagtacaaaaaagaacaagaacgagagaaagaaaaagaaaagcaaaaagatgacgaccacagtggtttagatgaagtataa

SEQ ID NO: 21 - DNA, 984 bp, Staphylococcus aureus
atgaaaaaatggcaatttgttggtactacagctttaggtgcaacactattattaggtgcttgtggtggcggtaatggtggcagtggtaatagtgatttaaaaggggaagctaaaggggatggctcatcaacagtagcaccaattgtggagaaattaaatgaaaaatgggctcaagatcactcggatgctaaaatctcagcaggacaagctggtacaggtgctggtttccaaaaattcattgcaggagatatcgacttcgctgatgcttctagaccaattaaagatgaagagaagcaaaaattacaagataagaatatcaaatacaaagaattcaaaattgcgcaagatggtgtaacggttgctgtaaataaagaaaatgattttgtagatgaattagacaaacagcaattaaaagcaatttattctggaaaagctaaaacatggaaagatgttaatagtaaatggccagataaaaaaataaatgctgtatcaccaaactcaagtcatggtacttatgacttctttgaaaatgaagtaatgaataaagaagatattaaagcagaaaaaaatgctgatacaaatgctatcgtttcttctgtaacgaaaaacaaagagggaatcggatactttggatataacttctacgtacaaaataaagataaattaaaagaagttaaaatcaaagatgaaaatggtaaagcaacagagcctacgaaaaaaacaattcaagataactcttatgcattaagtagaccattattcatttatgtaaatgaaaaagcattgaaagataataaagtaatgtcagaatttatcaaattcgtcttagaagataaaggtaaagcagctgaagaaggtggatatgtagcagcaccagagaaaacatacaaatcacaattagatgatttaaaagcatttattgataaaaatcaaaaatcagacgacaagaaatctgatgataaaaagtctgaagacaagaaataa

SEQ ID NO: 22 - DNA, 1074 bp, Staphylococcus aureus
atgaaaggtaaatttttaaaagttagttctttattcgttgcaactttgacaacagcgacacttgtgagttctccagcagcaaatgcgttatcttcaaaagctatggacaatcatccacaacaaacgcagacagacaaacagcaaacacctaagattcaaaaaggcggtaaccttaaaccattagaacaacgtgaacgcgctaatgttatattaccaaataacgatcgtcaccaaatcacagatacaacgaatggtcattatgcacctgttacttatattcaagttgaagcacctactggtacatttattgcttctggtgtagttgtaggtaaagatacacttttaacaaataaacacatcgtagatgctacgcacggtgatcctcatgctttaaaagcattcgcttctgcaattaaccaagacaattatcctaatggtggtttcactgctgaacaaatcactaaatattcaggcgaaggtgatttagcaatcgttaaattctcccctaatgagcaaaacaaacatattggcgaagtagttaaaccagcaacaatgagtaataatgctgaaacacaagttaaccaaaatattactgtaacaggatatcctggtgataaacctgtcgcaacaatgtgggaaagtaaaggaaaaataacgtacttaaaaggtgaagcaatgcaatatgatttaagtacaactggtggtaactcaggttcacctgtatttaatgaaaaaaatgaagtcattggcattcattggggtggcgttccaaatcaatttaacggtgcagtatttattaatgaaaatgtacgcaacttcttaaaacaaaatattgaagatatcaatttcgcaaatgatgaccaccctaacaaccctgataatccagacaatccaaataatccggacaatcctaacaaccctgataaccctaacaaccctgataatccagacaatcctaataatcctgataaccctaacaacccggacaatccaaataaccctgaccaacctaacaacccaaataacccggacaatggcgataacaataattcagacaaccctgacgctgcataa

SEQ ID NO: 23 - DNA, 1200 bp, Staphylococcus aureus
atgaagcgtacattagtattattgattacagctatctttatactcgctgcttgtggtaaccataaggatgaccaggctggaaaagataatcaaaaacataacaatagttcaaatcaagtaaaagaaattgctacggataaaaatgtacaaggtgataactatcgtacattgttaccatttaaagaaagccaggcaagaggacttttacaagataacatggcaaatagttataatggcggcgactttgaagatggtttattgaacttaagtaaagaagtgtttccaacagacaaatatttgtatcaagatggtcaatttttggacaagaaaacaattaatgcctatttaaatcttaagtatacaaaacgtgaaatcgataaaatgtctgaaaaagataaaaaagacaagaaagcgaatgaaaatttaggacttaatccatcacacgaaggtgaaacagatcctgaaaagattgcagaaaaatcaccagcctatttatctaacattttagagcaagatttttatggtggtggagatacaaaaggtaagaatattaaaggtatgacgattggtttagctatgaatagtgtttattactataaaaaagaaaaagatggaccgacttttagtaaaaaactagatgatagcgaagttaaaaagcaaggtaaacaaatggctagtgagatattatcaaggttacgtgaaaatgatgatttaaaagatataccaattcattttgcaatttataagcaatcaagtgaagattcaatcacaccaggtgaatttatcactcaagcgactgcagaaaagagtcaaacaaagcttaatgaatggcataatatcaatgaaaaatcagctttattaccttcttcaacagcagcagattatgatgaaaatttaaataataatttcaagcaatttaatgataatttgcaatcatatttttctaatttcacacaagcagtaggaaaagttaaatttgttgataaaaagccacaacgattagtagtagatttaccaatcgattactatggacaagctgaaacaattggtattacacagtacgttactgaacaagcgaataaatatttcgataaaatcgataactatgaaattcggattaaagatggtaaccaaccacgtgctttaattagtaagacaaaagatgacaaagaaccgcaagttcatatttacagtaattaa

SEQ ID NO: 24 - DNA, 1488 bp, Staphylococcus aureus
atgagggaaaattttaagttacgtaaaatgaaagtcgggttagtatctgttgcaattacaatgttatatatcatgacaaacggacaagcagaagcatcagaggctaatgagaagccaagtacaaatcaagaatcaaaagttgtttcacagactgaacaaaattcaaaagaaacaaaaacagtagaatctaataagaactttgttaaattagatactattaaacctggagctcaaaagataacgggaactactttaccaaatcactatgttttattaacagttgatgggaaaagtgcggattcagtagaaaatggcggtttgggttttgttgaagcaaatgacaaaggagaatttgagtaccctttaaataatcgtaaaattgttcataatcaagaaattgaggtttcgtcgtcaagccctgatttaggtgaagatgaagaagatgaagaggtggaagaagcttcaactgataaagctggcgttgaggaagaaagtacagaagctaaagttacttacacaacaccgcgatatgaaaaagcgtatgaaataccgaaagaacaactaaaagaaaaagatggacatcaccaagtttttatcgaacctattactgaaggatcaggtattattaaagggcatacgtctgtaaaaggtaaagttgctttatctattaataataaatttattaattttgaagagagcgttaagggcggagttagtaaagaagacactaaagctagttcagatggtatctggatgcctattgatgacaaaggatactttaactttgacttcaaaacgaaacgtttcgataatttagagttaaaagaaggtaatgacatttcactaacatttgcacctgatgatgaagaagatgcattaaaacctttaattttcaaaactaaagtaacgagcttagaagatatcgataaagcagaaactaaatatgaccatactaaactcaacaaagtgaaagttttagataatgttaaagaagatttacatgttgatgaaatatatggaagcttatatcatacagacaaaggtaaaggtattcttgataaagaaggtactaaagtaattaaaggaaagactaaattcgcgaatgcagtagtgaaggtagactctgaactaggtgaagcacaattattccctgatttacaagtaaatgaaaaaggtgaatttagctttgactcacatggtgctggttttagattacaaaatggagaaaaattaaacttcacagtggttgatcctattacaggtgacttgttaagtaatgagtttgtttctaaagagattgatattgaagaaacacctgaacaaaaagcggatcgtgagtttgacgaaaaacttgaaaatacgcctgcttactacaagttatacggcgataaaatagttggattcgatactaacgatttcccgattacttggttctatccattgggtgaaaagaaagttgaacgtacaacacctaaattagaaaaataa

SEQ ID NO: 25 - DNA, 1524 bp, Staphylococcus aureus
atgtctaaaaagttaaaaattataattcctattattattgtcttattattaataggtggaatcgcatggggagtttatgcattttttgcaaacacaccgaaaaatacatacttaaaaagtgaacaacaaactgcaaaaatgtataaagattattttaatgaccgttttgaaaacgaagtgaagttccaagaaaagatgaaagataattcatttttatcttcattagaattaagcgcagatgcatctgatgaaattgttaaagggcttggtattcctaaatctgttgttaatgcttcgaaaattaaaatgtcatatggacatgatcctaaaaaagagaaatcaatgattaatcttgaaccaacaatagcagactctgcattagggaaattccagttagctgcagataaagataagcattatttcgaatcaccattatttaaagggaaatatagtgttaataattctgatttattatcaacttattcaaaacttacaggtgaagatgaagaaacagcaaaagaaaatggtattacaaaccaacaactaaatttaaatactcttttcagtaatgctcaagcacaacaaagtgactacagcaaaattgccgaaaaatattccgaacttattgtcgacaaattagatgacgataattttgataaaggtaaaaaagaagaaattaaggttaatggtgaaaagtacaaagttagacctgtcacgttaacacttagcagagctgacactaaaaaaattacattagctgtattagaagaagctaaaaaggataaagaccttaaaaaattaatggaagaacaaggtactacaaaagactttgaaaaagacattaaaaaagcaattgacgatgtcaaagaaactaaaaaggatgaatttgctaaaattcaatctaaaatttataccgaaaaacatacgattgtaaaacgagaaattactattacagacaaagaaaataataaaactaaaatcaaaggtactaatactttagaagacgataagttaaaactagattacgcacttgatttcgatcaagataaatacacgtatgctgaagcgaaatatacaattaaaggcgtatcttctaaggaaaaagacaataaatacagtgataaatacgaatttggtaaaaagacagaatatgatgaatcaaaaatcaaattagataaccaagaaaaagtagatggcacaaaacgtcaagataaaggtaaaatcactgtcgcgttagataaatatagcgacgaaaatgaattcacttttgaaaataatatagattctgacgtaaaaaataacactcagaaatctacgttaaatatcggcatcaaatatgctgaagaaccaattaatttcattttaaaatctagcacaaaattgaaagcagatattgattttgatgatagtggtgcgaaagatttcaatagtctatcttcaaaagaccgtgaaaaacttgaaaaagaaatcgaaaaaaatggcggcaaaatgtttgaatcaattttaaaaaaggcatctaaataa

SEQ ID NO: 26 - DNA, 1530 bp, Staphylococcus aureus
gtgaggaaattttcaagatatgcatttacaagtatggcaacagtaacgttgctgagctctttgacacctgcagcactagcgagtgatacgaatcacaaaccagcaacttcagatattaattttgaaatcacgcaaaagagtgatgcagttaaagcattaaaagagttacctaaatctgaaaatgtgaaaaatcattatcaagattactctgttacagatgtaaaaacagataagaaaggattcacgcattacacgttacaaccgagtgtggatggtgtgcatgcgcctgacaaagaagtgaaagtgcatgcggacaaatcgggtaaagtcgttttaatcaacggtgatactgatgcgaagaaagtaaagccgacaaataaagtgacattaagcaaggatgaagcggctgacaaagcatttaacgcagttaagattgataaaaataaagctaaaaacctccaagatgacgttatcaaagaaaataaagtcgaaatcgatggtgacagtaataaatacatttacaatattgaattaattacagtaacaccagaaatttcacattggaaagttaaaattgatgcagacacaggagcagttgttgaaaaaacgaacttagttaaagaagcagcagcaactggcacaggtaaaggtgtgcttggagatacaaaagatatcaatatcaatagtattgatggtggatttagtttagaggatttgacgcatcaaggtaaattatcagcatacaattttaacgatcaaacaggtcaagcgacattaattactaatgaagatgaaaacttcgtcaaagatgatcaacgtgctggtgtagatgcgaattattatgctaaacaaacatatgattactacaaaaatacatttggtcgtgagtcttacgataaccatggtagtccaatagtctcattaacacatgtaaatcattatggtggacaagataacagaaataacgctgcatggattggagacaaaatgatttatggtgatggcgatggccgcacgtttacaaatttatcaggtgcaaatgacgtagtagcacatgagttaacacatggcgtgacacaagaaacggcgaatttagagtataaagatcaatctggtgcgttaaatgaaagcttttcagatgtttttggatactttgtagatgatgaggatttcttgatgggtgaagatgtttacacaccaggaaaagagggagatgctttacgaagcatgtcaaacccagaacaatttggtcaaccatctcatatgaaagactatgtatacactgaaaaagataacggtggtgtgcatacgaattctggcattccaaataaagcagcttataacgtaattcaagcaatagggaaatctaaatcagaacaaatttactaccgagcattaacggaatacttaacaagtaattcaaacttcaaagattgtaaagatgcattataccaagcggctaaagatttatatgacgagcaaacagctgaacaagtatatgaagcatggaacgaagttggcgtcgagtaa

SEQ ID NO: 27 - DNA, 1548 bp, Staphylococcus aureus
atgaaaaagaaattaggtatgttacttcttgtaccagccgtaactttatcattagccgcatgtgggaatgatgatggaaaagataaagatggcaaggtaacaattaaaacgacagtttatccattgcaatcatttgcagagcaaattggtggaaaacacgtgaaggtatcatcaatctatccagcagggacagatttacatagctatgaaccaacacaaaaagatatattaagtgcaagcaagtcagacttgtttatgtatacaggggataatttagatccggttgctaagaaagttgcatctactattaaagataaagataaaaaactgtctttagaagataaattagataaagcaaagcttttaactgatcaacacgaacatggtgaagagcatgaacatgagggacatgatcatgggaaagaagaacatcatcatcatggcggatatgatccacacgtatggttagatcctaaaattaaccaaactttcgctaaagaaattaaagatgaattagtgaagaaagatccaaaacataaagatgactatgagaaaaactacaaaaaattaaacgacgatcttaagaaaattgataacgatatgaagcaagttactaaagataagcaaggtaatgcagtattcatttcacatgaatcaattggatacttagctgatcgttatggttttgttcaaaaaggtattcaaaacatgaatgctgaagatccatcacaaaaagaattgactaaaattgttaaagaaattagagatagcaatgctaaatatattctttacgaagataatgttgcgaataaagtgactgaaacaattcgtaaagaaacagatgcgaagcctttaaaattctacaacatggagtctttaaataaagaacaacagaaaaaagataatattacctatcaatcattaatgaaatcgaatattgaaaatatcggtaaagctttagacagtggtgttaaagtgaaagacgacaaagctgaaagtaaacacgacaaagcaatttctgatgggtattttaaagatgagcaagttaaagaccgtgaattaagcgattatgctggtgaatggcaatctgtttacccttacttaaaagacggtacgcttgatgaagtgatggaacataaagctgaaaatgatccgaagaaatctgctaaagatttaaaagcttattatgacaaaggatataaaactgatattactaacattgatataaaaggaaatgaaattacatttactaaagatggtacgaaacacactggtaaatatgaatacaatggtaagaaaacattgaaatatcctaaaggtaaccgtggcgtgagatttatgtttaaattggtcgatggtaatgataaagacttaccgaaattcatccaatttagcgatcacaacattgcacctaaaaaggcagaacacttccatatctttatgggtaatgataatgacgcgttattaaaagaaatggataactggccaacatattatccttcaaaattaaataaagaccaaatcaaagaagaaatgttagcgcattaa

SEQ ID NO: 28 - DNA, 1695 bp, Staphylococcus aureus
atggtgttatatatcattttggcaataattgtgattatattgattgctgtaggtgtattattctatttacgttcaaataaaagacaaataatagaaaaagcaatcgaacgtaaaaatgaaattgaaacgttaccttttgatcaaaaccttgcacaattatctaagttgaatttaaaaggtgaaacaaaaacgaaatacgatgcaatgaaaaaggacaacgtagaaagtacaaataagtatctagctcctgtggaagaaaaaatccataatgctgaggctttattagataaatttagtttcaacgcatctcaatgtgaaattgatgatgcaaatgagttgatggatagttacgaacaaagctatcagcaacaattagaagatgtaaatgaaattattgcgttatacaaagataatgatgaattatatgacaaatgtaaggttgattatcgtgaaatgaaacgtgatgttttagcaaatcgtcatcaatttggtgaggcagcaagtcttcttgaaactgaaattgaaaaattcgagccaaggttagagcaatatgaagtactaaaagctgatggtaattatgtacaagcgcacaaccatatagctgccttgaatgaacaaatgaaacagctaagatcttatatggaagaaataccagaattaattagagaaactcaaaaagaattacctggtcaattccaagatttaaaatatggttgccgtgatcttaaagttgaagggtatgatctggatcacgtaaaagtagacagtacattacaaagcttaaaaacagagcttagtttcgttgaaccattaattagtcgcttagaattagaagaagctaatgataaactagctaatatcaatgataagttagatgacatgtatgatttaattgaacatgaagttaaagctaaaaatgatgtcgaagaaacaaaagatatcattacggataacttattcaaagcaaaagacatgaattatacattgcaaacagaaattgaatatgtacgtgaaaactactatataaatgaatctgatgctcagagtgttcgtcaatttgaaaatgaaattcaaagtttaatttctgtatatgatgatattttaaaagaaatgtctaaatctgctgtacgatatagcgaggttcaggataatttacaatatttagaagatcatgtcacagttattaatgacaaacaagaaaagctacaaaatcatctgattcaattgcgtgaagatgaagcagaagcagaagacaatctgttacgagtacaatcgaagaaagaagaagtgtatcgtcgattacttgcttctaacttaacaagcgttcctgaaaggtttatcatcatgaaaaatgaaattgatcatgaagttcgtgatgttaacgaacaatttagtgaacgtccaatacacgttaaacagttaaaagataaagtgtctaaaattgtgattcaaatgaatacatttgaagatgaagcaaatgatgttcttgttaatgctgtttatgcagagaaattaattcaatatggaaatagatatcgtaaggactatagcaatgttgataagagcttaaatgaagctgaacgattatttaaaaataatcgctataagcgtgcgattgaaattgcagagcaagctcttgaaagtgttgagccaggtgtcactaaacatattgaagaagaagttattaagcaatag

SEQ ID NO: 29 - DNA, 1860 bp, Staphylococcus aureus
atgcctaaaaataaaattttaatttatttgctatcaactacgctcgtattacctactttagtttcacctaccgcttatgctgacacacctcaaaaagatactacagctaagacaacatctcatgattccaaaaaatctactgatgatgaaacttctaaggatactacaagtaaagatattgataaagcagacaacaataatactagtaaccaagacaataacgacaaaaaagttaaaactatagacgacagcacttcagactctaacaatatcattgattttatttataagaatttaccacaaaccaatataaaccaattgctaaccaaaaataaatacgatgataattactcattaacaactttaatccaaaacttattcaatttaaattcggatatttctgattacgaacaacctcgtaatggtgaaaagtcaacaaatgattcgaataaaaacagtgataatagcatcaaaaatgatacggatacgcaatcatctaaacaagataaagcagacaatcaaaaagcacctaaatcaaacaatacaaaaccaagtacatctaataagcaaccaaattcgccaaagccaacacaaccaaatcaatcaaatagtcaaccagcaagtgacgataaagtaaatcaaaaatcttcatcgaaagataatcaatcaatgtcagattcggctttagattctattttggatcaatacagtgaagatgcaaagaaaacacaaaaagattacgcatctcaatctaaaaaagacaaaaatgaaaaatctaatacaaagaatccacagttaccaacacaagatgaattgaaacataaatctaaacctgctcaatcattcaataacgatgttaatcaaaaggatacacgtgcaacatcactattcgaaacagatcctagtatatctaacaatgatgatagtggacaatttaacgttgttgactcaaaagatacacgtcaatttgtcaaatcaattgctaaagatgcacaccgcattggtcaagataacgatatttatgcgtctgtcatgattgcccaagcaatcttagaatctgactcaggtcgtagtgctttagctaagtcaccaaaccataatttattcggtatcaaaggtgcttttgaagggaattctgttccttttaacacattagaagctgatggtaatcaattgtatagtattaatgctggattccgaaaatatccaagcacgaaagaatcactaaaagattactctgaccttattaaaaatggtattgatggcaatcgaacaatttataaaccaacatggaaatcggaagccgattcttataaagatgcaacatcacacttatctaaaacatatgctacagatccaaactatgctaagaaattaaacagtattattaaacactatcaattaactcagtttgacgatgaacgtatgccagatttagataaatatgaacgttctatcaaggattatgatgattcatcagatgaattcaaacctttccgcgaggtatctgataatatgccatatccacatggccaatgtacttggtacgtatataaccgtatgaaacaatttggtacatctatctcaggtgatttaggtgatgcacataattggaataatcgagctcaataccgtgattatcaagtaagtcatacaccaaaacgtcatgctgctgttgtatttgaggctggacaatttggtgcagatcaacattacggtcatgtagcatttgttgaaaaagttaacagtgatggttctatcgttatttcagaatccaatgttaaaggattaggtatcatttctcatagaactatcaatgcagctgccgctgaagaattatcatatattacaggtaaataa

SEQ ID NO: 30 - DNA, 2046 bp, Staphylococcus aureus
atgatgaaaagtcaaaataagtatagtattcgtaaatttagtgtaggtgcatcttccattttaatagctacattactatttttaagtggtggacaagcacaagcagctgagaagcaagtgaatatgggaaattcacaggaggatacagttacagcacaatctattggggatcaacaaactagggaaaatgctaattatcaacgtgaaaacggtgttgacgaacagcaacatactgaaaatttaactaagaacttgcataatgataaaacaatatcagaagaaaatcatcgtaaaacagatgatttgaataaagatcaactaaaggatgataaaaaatcatcgcttaataataaaaatattcaacgtgatacaacaaaaaataacaatgctaatcctagggatgtaaatcaagggttagaacaggctattaatgatggcaaacaaagtaaagtggcgtcacagcaacagtcaaaagaggcagataatagtcaagacttaaacgctaataacaatctaccttcacaaagtcgaacaaaggtatcaccatcattaaataagtcagatcaaacaagtcaacgagaaattgttaatgagacagaaatagagaaagtacaaccgcaacaaaagaatcaagcgaatgataaaattactgaccacaattttaacaatgaacaagaagtgaaacctcaaaaagacgaaaaaacactatcagtttcagatttaaaaaacaatcaaaaatcaccagttgaaccaacaaaggacaatgacaagaaaaatggattaaatttattaaaaagtagtgcagtagcaacgttaccaaacaaagggacaaaggaacttactgcaaaagcgaaaggtgatcaaacgaataaagttgccaaacaagggcagtataaaaatcaagatcctatagttttagtgcatggtttcaatgggtttacagatgatattaatccttcagtgttagctcattattggggcggtaataaaatgaacattcgccaagatttagaagaaaatggttacaaagcttatgaagcaagtataagtgcttttggaagtaactatgaccgcgcagttgaactttattattatatcaaaggcggtcgtgtagattatggtgcagcacatgcagcaaaatatggacatgaacgttatggaaaaacatacgaaggaatttacaaagactggaaaccaggacagaaggtacaccttgttggacatagtatgggtggtcaaacgatacgtcaactagaagaattactgcgtaatggtagtcgtgaagaaatagagtatcaaaagaaacatagtggcgaaatttctccactattcaaaggtaataatgacaatatgatttcatcaattactactttaggaacgccacataatggaacgcatgcttcagatttagctggtaatgaagctttagtgagacaaattgtatttgatatcggtaaaatgtttggtaataaaaattcaagagtagacttcgggttggctcaatggggtctaaaacagaagccaaatgaatcatatattgattatgtcaaacgcgttaaacaatctaatttatggaaatcaaaagataatggattttacgatctgacgcgtgagggtgcaacagatttaaatcgtaaaacgtcgttgaaccctaacattgtgtataaaacatacactggtgaagcaacgcacaaagcattaaatagcgatagacaaaaagcagacttaaatatgtttttcccatttgtgattactggtaacttaatcggtaaagctactgaaaaagaatggcgagaaaacgatggtttagtatccgttatttcttctcaacatccatttaatcaagcttatacaaatgcgacggataaaattcaaaaaggcatttggcaagtaacgcctacaaaacatgattgggatcatgttgattttgtcggacaagatagttctgatacagtgcgcacaagagaagaattacaagatttttggcatcatttagcagacgatttagtgaaaactgaaaaggtgactgatactaagcaagcataa

SEQ ID NO: 31 - DNA, 2421 bp, Staphylococcus aureus
atgacaaataaaatgaagaaatggcaaaaattatccaccattacgttattaatgaccggagtgattgctttaaataatggtgaatttagaaatgttgataaacatcaaatcgctgtggctgatacgaatgttcaaacgccagattatgaaaaattgaagaagacgtggctcgacgttaactacggttatgatcagtatgatgagaataatcaagatatgaagaagaagtttgatgctaaagaaaaagaagccaagaagttacttgatgacatgaaaactgatacgaatagaacatatttgtggtcaggagctgaaaaccttgaaactaattcttctcacatgacaaaaacctatcgtaatatcgagaaaatcgcagaatcaatgcaacataagaatacggtattaaaaacagttgaaaacaagttgaaaataaaagaagccctagattggatgcacaaaaatgtttatggcaagaatccttctcaaaaagtcgaggatttaactaaaaatcgtaaggggcaaactacacccaagaataactcattgaattggtgggattatgaaattggtacgccaagagcattaacaaatacactacttctaatggatgatatgctcactaaagatgaaatgaaaaattattcaaaacctattagtacatatgcaccatccagtgacaaaattttatcttctgttggtgaatcagaagatgctaaaggtggaaatttagtggacatttctaaagtaaaacttttagaaagtgttattgaagaagatgtagatatgttgaaaaagtctatagattcttttaataaagtgttcacttatgttcaagattctgccactggtaaaggtcgcaatggattctataaagatggctcttacattgatcatcaagatgtcccttacactggtgcttatggtgttgtactattagagggtatttctcaaatgatgccgatgataaaagaatctccttttaaaactacacaagataatgctacattaagcaattggattgacgaagggtttatgccattaatctataaaggtgaaatgatggatttatcacgaggtagagctatcagtcgtgaaaatgaaacgagtcatacagcgtcagcgactgtaatgaaatcattgttgagattgaatgataccatggatgattcaacaaaaactagatataagcaaatcgttaaaacttctgttaattctgattcaagttacaaccaaaataattatttaaattcatattcagacatagctaaaatgaaaaagttaatgaatgatagtactatttctaaaaacgatttaacacagcaacttaaaatatataatgacatggatcgtgtcacctatcacaataaagacctggactttgcatttggtttaagtatgacatcgaaaaacatcgcacgatacgaaaatatcaacggagagaacttaaaaggttggcacaccggtgcaggcatgtcttatttatataacagcgatgtcaaacactatcgcgataacttctgggcaacagccgatatgacttgtcttccaggcactactactttaaatgatatgccatctactaatactaagaatgataaatcttttgttggcgggacaaaattaaataataaatacgcaagcatcggtatggattttgaaaatcaggacaaaactttaactgccaaaaaatcatatttcatattaaacgataaaattgtcttcttaggaactggcattaaaagtactgattcatcaaagaatccagttacaagtgttgaaaatcgcaaagcaaatgggtataaattatttaaagatgatattgaaattaccacttcagatgttaatgctcaggaaacccattcagtctttttagagtccaacgatactaaaaagaacattggttatcatttcttagacaagccaaaaataactgtaaaaaaagaaagtcatactggtaagtggagtgaaattaataaaagtcaaaaaaaagatgacaaaaaagatgagtattatgaagtaactcaaacacataatacatctgacagtaaatatgcatatgttttgtatcctggtttatcaaaaagtgattttaaatcgaagaataataatgtaagtattgttaaacaagatgaagattttcatgtgataaaagataatgatggcgtatttgctggggttaattatagtgataatactaaatcttttgatataaacggaattactgttgaattaaaagaaaaaggcatgtttgtaattaaaaagaaagatgataaagcatataaatgtagcttctataatcctgaaactacaaataccgcttcaaatatagaatcaaaaatttttattaaaggttacaccataactaataaaagtgtcataaactctaatgatgctggtgtaaactttgaattaactaaataa

SEQ ID NO: 32 - DNA, 2427 bp, Staphylococcus aureus
atgacatatagaatgaagaaatggcaaaaattgtccaccattacgttattaatggctggtgtgattactttgaatggtggtgaattcagaagtattgataaacatcaaatcgctgtggctgatacgaatgttcaaacgacagattatgaaaagttgaggaacatatggctggacgttaactatggttatgataagtatgatgagaataatccagatatgaagaagaagtttgaggctacggagaatgaggcagagaaattactcaaggaaatgaaaactgaaagtgataggaaatacttgtgggaaagctcaaaagatttagatacgaagtctgcggatatgactcgtacctatcgtaatattgagaaaatctcagaagcgatgaaacataaaaatactaaattaaaaacagatgaaaacaagacaaaagtaaaagatgcacttgagtggctgcataaaaatgcatatggaaaagaaccagataaaaaagttgctgatttgacctcaaactttaaaaataaaacttctagaaataccaacttaaattggtgggattatgaaattggaacacctagagcattaacaaatacgcttatactcttacaagaagatttcactgatgaagaaaagaaaaaatatacagctcctattaaaactttcgccccagatagtgacaaaatattatcttctgtaggaaaatctgaacctgctaaaggcggaaatttagtagacatttctaaagtaaaacttttagaaagtattatcgaagaagacaaagatatgatgaaaaagtctatagattcatttaatacagtcttcacttacgcgcaaaattctgccactggaaaagaacgtaatggattctataaagatggctcttacattgatcatcaagacgtcccatacactggtgcttatggcgttgtactattagagggtatttctcaaatgatgccgatgataaaagaaacaccttttaatgatagtaaccaaaatgatacaaccttaaaatcatggattgacgacggatttatgccactcatttataaaggtgaaatgatggatttatcaagaggtagagctatcagtcgtgaaaatgaaacgagtcactcagcatctgcaacagtaatgaaatcattgttgagattgagtgataccatggataagtctacaaaagctaaatataaaaagattgtcaagacttcagtagagtcagattcaagttataaacaaaccgattatttaagctcttattcggatataagcaaaatgaagtctttaatggaagacagcactatttctactaacggtttaacacaacaacttaaaatatataatgacatggatcgtgtcacctatcacaataaaggcttagactttgcatttggtttaagtatgacgtcgaaaaacgtcgcacgttacgaaagtatcaacggagagaacttaaaaggttggcacactggtgctggaatgtcttatttatacaatagcgatgtgaaacactaccgtgataacttctgggcgacagctgatatgaaacgtttagcaggtactacaactttagataatgaagaacctaaaagtacggatgttaaaaagtctagtaaaacttttgtaggaggaacaaaattcgatgaccaacatgctagtatcggaatggattttgaaaatcaggacaaaactttaactgccaaaaaatcatatttcatattaaacgataaaattgtcttcttaggaactggcattaaaagtactgattcatcaaagaatccagttacaacgattgaaaatcgcaaagcgaatgattataaattatataaagatgatacgcaaacaaccaattccgataatcaggaaaccaattccctctttttagagtcaacgaatagcactcaaaacaatataggttatcattttttaaacgaatcgaaaataactgtaaaaaaagaaagtcatactggtaagtggagtgatataaataaaagccaaaaggatatacaaaaaactgatgagtattatgaagtaactcaaaagcattctaatacagatagtaaatatgcatatgtgttgtatccaggcttatctaaagatgtctttaaatccaaagcaagcaaagtaactgtcgttaagcaagaagatgacttccacgttgtgaaagataatgaatcggtttgggctggtatcaattatagtgatagcgctaaaacttttgaaattaataacactaaagtcgaagttaaagccaaaggaatgtttattcttacaaagaaagatgataacacttatgaatgtagcttctataatcccgaatctacaaattccgtttcagatattgaatctaaaatttcaatgactggatactctattataaacaaaaatacgtcgacttctaatgaatccggcgtacgctttgaattaactaaataa

SEQ ID NO: 33 - RNA, 423 nt, Staphylococcus aureus
auggcaaaagguaauuuauuuaaagcgauuuuagguauagguggcgcuguagcagcuguacuuguuacacguaaagauagucgugacaagcugaaagcagaauauaauaaauacaaacaagauccucaaagcuauaaagauaaugcuaaggauaaagcgacgcaauuaggaacaauugcaaaugaaacaauuaaagaaguaaaaacaaauccgaaagaauaugcuaauagauuaaaaaauaauccaaaagcauuuuucgaagaagaaaaaucaaaauuuaccgaauaugacaauaagacugacgaaaguauugaaaaagguaaauuugaugaugaagguggcgcagcaccaaauaauaauuuacguaucgucacugaagaagauuuaaaaaagaauaaaaaugcauugucugauaaagaauaa

SEQ ID NO: 34 - RNA, 582 nt, Staphylococcus aureus
augaaaaaauugguuucaauuguuggcgcaacauuauuguuagcuggauguggaucacaaaauuuagcaccauuagaagaaaaaacaacagauuuaagagaagauaaucaucaacucaaacuagauauucaagaacuuaaucaacaaauuagugauucuaaaucuaaaauuaaagggcuugaaaaggauaaagaaaauaguaaaaaaacugcaucuaauaauacgaaaauuaaauugaugaauguuacaucaacauacuacgacaaaguugcuaaagcuuugaaauccuauaacgauauugaaaaggauguaaguaaaaacaaaggcgauaagaauguucaaucgaaauuaaaucaaauuucuaaugauauucaaagugcucacacuucauacaaagaugcuaucgaugguuuaucacuuagugaugaugauaaaaaaacgucuaaaaauaucgauaaauuaaacucugauuugaaucaugcauuugaugauauuaaaaauggcuaucaaaauaaagauaaaaaacaacuuacaaaaggacaacaagcguugucaaaauuaaacuuaaaugcaaaaucauga

SEQ ID NO: 35 - RNA, 630 nt, Staphylococcus aureus
augaaaaaauuaguuacaggguuauuagcauuaucauuauuuuuagcugcauguggucaagauagugaccaacaaaaagacaguaauaaagaaaaagaugauaaagcgaaaacugaacaacaagauaaaaaaacaaaugauucaucuaaagauaagaaagacaauaaagaugauaguaaagacguaaacaaagauaauaaagauaauagugcaaacgauaaccagcaacaaucuaauucaaaugcaacaaacaaugaccaaaaucaaacgaauaauaaccagucaaacaguggacaaacgacuaacaaucaaaaaucaaguuacguugcaccauauuauggacaaaacgcagcgccaguggcucgucaaauuuauccauuuaaugguaauaaaucacaagcauuacaacaauugccuaauuuccaaacagcuuuaaaugcagcuaacaacgaagcaaauaaauuugguaauggucauaaaguuuauaaugauuauucaauugaagaacauaaugguaacuauaaguauguuuuuaguuuuaaagacccaaacguaaauggaaaauauucaauuguaacgguugauuauacuggacaagcaaugguuacugauccaaacuaccaacaauaa

SEQ ID NO: 36 - RNA, 729 nt, Staphylococcus aureus
augaaaaaaguaauggggauauuauuagcaaguacacuuaucuuaggugcuuguggacaucaucaagauagugcaaaaaaagagagcacuagucacaaaaagaaagaaaaugacaaugaagaauuaaaugaagaacuuaaagaauuuaaaagcaaaaaaaauauggauauaaaaauuaaaggcgauacuauuguuagugacaaauuugaagcuaaaauaaaagaaccguuuaucaucaaugaaaaagaugagaaaaagaaauauaucgcuuuuaaaauggaaauuacugcuaaaaaagacgauaaagauuuaaauccaucuucuauuucucaugacuauauuaauaucacucaagaugauaaaaauacaguaaauaaauuaagagaugguuaucuuuuaagugauaaaaauuauaaagauuggacagaacauaaccaagaucaaauuaaaaaaggcaaaacugcacaagccauguuuaucuaugaguuaagaggugauggaaacauuaauuuaaauguccauaaauacucagaagauaaaacaguugauucuaaaucauucaaauuuaguaaacuuaaaaccgaagauuuuucucauagagcggaaacaagggaagaaguagaaaagaaagaaaaagaauuugaagaagaguacaaaaaagaacaagaacgagagaaagaaaaagaaaagcaaaaagaugacgaccacagugguuuagaugaaguauaa

SEQ ID NO: 37 - RNA, 984 nt, Staphylococcus aureus
augaaaaaauggcaauuuguugguacuacagcuuuaggugcaacacuauuauuaggugcuugugguggcgguaaugguggcagugguaauagugauuuaaaaggggaagcuaaaggggauggcucaucaacaguagcaccaauuguggagaaauuaaaugaaaaaugggcucaagaucacucggaugcuaaaaucucagcaggacaagcugguacaggugcugguuuccaaaaauucauugcaggagauaucgacuucgcugaugcuucuagaccaauuaaagaugaagagaagcaaaaauuacaagauaagaauaucaaauacaaagaauucaaaauugcgcaagaugguguaacgguugcuguaaauaaagaaaaugauuuuguagaugaauuagacaaacagcaauuaaaagcaauuuauucuggaaaagcuaaaacauggaaagauguuaauaguaaauggccagauaaaaaaauaaaugcuguaucaccaaacucaagucaugguacuuaugacuucuuugaaaaugaaguaaugaauaaagaagauauuaaagcagaaaaaaaugcugauacaaaugcuaucguuucuucuguaacgaaaaacaaagagggaaucggauacuuuggauauaacuucuacguacaaaauaaagauaaauuaaaagaaguuaaaaucaaagaugaaaaugguaaagcaacagagccuacgaaaaaaacaauucaagauaacucuuaugcauuaaguagaccauuauucauuuauguaaaugaaaaagcauugaaagauaauaaaguaaugucagaauuuaucaaauucgucuuagaagauaaagguaaagcagcugaagaagguggauauguagcagcaccagagaaaacauacaaaucacaauuagaugauuuaaaagcauuuauugauaaaaaucaaaaaucagacgacaagaaaucugaugauaaaaagucugaagacaagaaauaa

SEQ ID NO: 38 - RNA, 1074 nt, Staphylococcus aureus
augaaagguaaauuuuuaaaaguuaguucuuuauucguugcaacuuugacaacagcgacacuugugaguucuccagcagcaaaugcguuaucuucaaaagcuauggacaaucauccacaacaaacgcagacagacaaacagcaaacaccuaagauucaaaaaggcgguaaccuuaaaccauuagaacaacgugaacgcgcuaauguuauauuaccaaauaacgaucgucaccaaaucacagauacaacgaauggucauuaugcaccuguuacuuauauucaaguugaagcaccuacugguacauuuauugcuucugguguaguuguagguaaagauacacuuuuaacaaauaaacacaucguagaugcuacgcacggugauccucaugcuuuaaaagcauucgcuucugcaauuaaccaagacaauuauccuaauggugguuucacugcugaacaaaucacuaaauauucaggcgaaggugauuuagcaaucguuaaauucuccccuaaugagcaaaacaaacauauuggcgaaguaguuaaaccagcaacaaugaguaauaaugcugaaacacaaguuaaccaaaauauuacuguaacaggauauccuggugauaaaccugucgcaacaaugugggaaaguaaaggaaaaauaacguacuuaaaaggugaagcaaugcaauaugauuuaaguacaacuggugguaacucagguucaccuguauuuaaugaaaaaaaugaagucauuggcauucauugggguggcguuccaaaucaauuuaacggugcaguauuuauuaaugaaaauguacgcaacuucuuaaaacaaaauauugaagauaucaauuucgcaaaugaugaccacccuaacaacccugauaauccagacaauccaaauaauccggacaauccuaacaacccugauaacccuaacaacccugauaauccagacaauccuaauaauccugauaacccuaacaacccggacaauccaaauaacccugaccaaccuaacaacccaaauaacccggacaauggcgauaacaauaauucagacaacccugacgcugcauaa

SEQ ID NO: 39 - RNA, 1200 nt, Staphylococcus aureus
augaagcguacauuaguauuauugauuacagcuaucuuuauacucgcugcuugugguaaccauaaggaugaccaggcuggaaaagauaaucaaaaacauaacaauaguucaaaucaaguaaaagaaauugcuacggauaaaaauguacaaggugauaacuaucguacauuguuaccauuuaaagaaagccaggcaagaggacuuuuacaagauaacauggcaaauaguuauaauggcggcgacuuugaagaugguuuauugaacuuaaguaaagaaguguuuccaacagacaaauauuuguaucaagauggucaauuuuuggacaagaaaacaauuaaugccuauuuaaaucuuaaguauacaaaacgugaaaucgauaaaaugucugaaaaagauaaaaaagacaagaaagcgaaugaaaauuuaggacuuaauccaucacacgaaggugaaacagauccugaaaagauugcagaaaaaucaccagccuauuuaucuaacauuuuagagcaagauuuuuauggugguggagauacaaaagguaagaauauuaaagguaugacgauugguuuagcuaugaauaguguuuauuacuauaaaaaagaaaaagauggaccgacuuuuaguaaaaaacuagaugauagcgaaguuaaaaagcaagguaaacaaauggcuagugagauauuaucaagguuacgugaaaaugaugauuuaaaagauauaccaauucauuuugcaauuuauaagcaaucaagugaagauucaaucacaccaggugaauuuaucacucaagcgacugcagaaaagagucaaacaaagcuuaaugaauggcauaauaucaaugaaaaaucagcuuuauuaccuucuucaacagcagcagauuaugaugaaaauuuaaauaauaauuucaagcaauuuaaugauaauuugcaaucauauuuuucuaauuucacacaagcaguaggaaaaguuaaauuuguugauaaaaagccacaacgauuaguaguagauuuaccaaucgauuacuauggacaagcugaaacaauugguauuacacaguacguuacugaacaagcgaauaaauauuucgauaaaaucgauaacuaugaaauucggauuaaagaugguaaccaaccacgugcuuuaauuaguaagacaaaagaugacaaagaaccgcaaguucauauuuacaguaauuaa

SEQ ID NO: 40 - RNA, 1488 nt, Staphylococcus aureus
augagggaaaauuuuaaguuacguaaaaugaaagucggguuaguaucuguugcaauuacaauguuauauaucaugacaaacggacaagcagaagcaucagaggcuaaugagaagccaaguacaaaucaagaaucaaaaguuguuucacagacugaacaaaauucaaaagaaacaaaaacaguagaaucuaauaagaacuuuguuaaauuagauacuauuaaaccuggagcucaaaagauaacgggaacuacuuuaccaaaucacuauguuuuauuaacaguugaugggaaaagugcggauucaguagaaaauggcgguuuggguuuuguugaagcaaaugacaaaggagaauuugaguacccuuuaaauaaucguaaaauuguucauaaucaagaaauugagguuucgucgucaagcccugauuuaggugaagaugaagaagaugaagagguggaagaagcuucaacugauaaagcuggcguugaggaagaaaguacagaagcuaaaguuacuuacacaacaccgcgauaugaaaaagcguaugaaauaccgaaagaacaacuaaaagaaaaagauggacaucaccaaguuuuuaucgaaccuauuacugaaggaucagguauuauuaaagggcauacgucuguaaaagguaaaguugcuuuaucuauuaauaauaaauuuauuaauuuugaagagagcguuaagggcggaguuaguaaagaagacacuaaagcuaguucagaugguaucuggaugccuauugaugacaaaggauacuuuaacuuugacuucaaaacgaaacguuucgauaauuuagaguuaaaagaagguaaugacauuucacuaacauuugcaccugaugaugaagaagaugcauuaaaaccuuuaauuuucaaaacuaaaguaacgagcuuagaagauaucgauaaagcagaaacuaaauaugaccauacuaaacucaacaaagugaaaguuuuagauaauguuaaagaagauuuacauguugaugaaauauauggaagcuuauaucauacagacaaagguaaagguauucuugauaaagaagguacuaaaguaauuaaaggaaagacuaaauucgcgaaugcaguagugaagguagacucugaacuaggugaagcacaauuauucccugauuuacaaguaaaugaaaaaggugaauuuagcuuugacucacauggugcugguuuuagauuacaaaauggagaaaaauuaaacuucacagugguugauccuauuacaggugacuuguuaaguaaugaguuuguuucuaaagagauugauauugaagaaacaccugaacaaaaagcggaucgugaguuugacgaaaaacuugaaaauacgccugcuuacuacaaguuauacggcgauaaaauaguuggauucgauacuaacgauuucccgauuacuugguucuauccauugggugaaaagaaaguugaacguacaacaccuaaauuagaaaaauaa

SEQ ID NO: 41 - RNA, 1524 nt, Staphylococcus aureus
augucuaaaaaguuaaaaauuauaauuccuauuauuauugucuuauuauuaauagguggaaucgcauggggaguuuaugcauuuuuugcaaacacaccgaaaaauacauacuuaaaaagugaacaacaaacugcaaaaauguauaaagauuauuuuaaugaccguuuugaaaacgaagugaaguuccaagaaaagaugaaagauaauucauuuuuaucuucauuagaauuaagcgcagaugcaucugaugaaauuguuaaagggcuugguauuccuaaaucuguuguuaaugcuucgaaaauuaaaaugucauauggacaugauccuaaaaaagagaaaucaaugauuaaucuugaaccaacaauagcagacucugcauuagggaaauuccaguuagcugcagauaaagauaagcauuauuucgaaucaccauuauuuaaagggaaauauaguguuaauaauucugauuuauuaucaacuuauucaaaacuuacaggugaagaugaagaaacagcaaaagaaaaugguauuacaaaccaacaacuaaauuuaaauacucuuuucaguaaugcucaagcacaacaaagugacuacagcaaaauugccgaaaaauauuccgaacuuauugucgacaaauuagaugacgauaauuuugauaaagguaaaaaagaagaaauuaagguuaauggugaaaaguacaaaguuagaccugucacguuaacacuuagcagagcugacacuaaaaaaauuacauuagcuguauuagaagaagcuaaaaaggauaaagaccuuaaaaaauuaauggaagaacaagguacuacaaaagacuuugaaaaagacauuaaaaaagcaauugacgaugucaaagaaacuaaaaaggaugaauuugcuaaaauucaaucuaaaauuuauaccgaaaaacauacgauuguaaaacgagaaauuacuauuacagacaaagaaaauaauaaaacuaaaaucaaagguacuaauacuuuagaagacgauaaguuaaaacuagauuacgcacuugauuucgaucaagauaaauacacguaugcugaagcgaaauauacaauuaaaggcguaucuucuaaggaaaaagacaauaaauacagugauaaauacgaauuugguaaaaagacagaauaugaugaaucaaaaaucaaauuagauaaccaagaaaaaguagauggcacaaaacgucaagauaaagguaaaaucacugucgcguuagauaaauauagcgacgaaaaugaauucacuuuugaaaauaauauagauucugacguaaaaaauaacacucagaaaucuacguuaaauaucggcaucaaauaugcugaagaaccaauuaauuucauuuuaaaaucuagcacaaaauugaaagcagauauugauuuugaugauaguggugcgaaagauuucaauagucuaucuucaaaagaccgugaaaaacuugaaaaagaaaucgaaaaaaauggcggcaaaauguuugaaucaauuuuaaaaaaggcaucuaaauaa

SEQ ID NO: 42 - RNA, 1530 nt, Staphylococcus aureus
gugaggaaauuuucaagauaugcauuuacaaguauggcaacaguaacguugcugagcucuuugacaccugcagcacuagcgagugauacgaaucacaaaccagcaacuucagauauuaauuuugaaaucacgcaaaagagugaugcaguuaaagcauuaaaagaguuaccuaaaucugaaaaugugaaaaaucauuaucaagauuacucuguuacagauguaaaaacagauaagaaaggauucacgcauuacacguuacaaccgaguguggauggugugcaugcgccugacaaagaagugaaagugcaugcggacaaaucggguaaagucguuuuaaucaacggugauacugaugcgaagaaaguaaagccgacaaauaaagugacauuaagcaaggaugaagcggcugacaaagcauuuaacgcaguuaagauugauaaaaauaaagcuaaaaaccuccaagaugacguuaucaaagaaaauaaagucgaaaucgauggugacaguaauaaauacauuuacaauauugaauuaauuacaguaacaccagaaauuucacauuggaaaguuaaaauugaugcagacacaggagcaguuguugaaaaaacgaacuuaguuaaagaagcagcagcaacuggcacagguaaaggugugcuuggagauacaaaagauaucaauaucaauaguauugaugguggauuuaguuuagaggauuugacgcaucaagguaaauuaucagcauacaauuuuaacgaucaaacaggucaagcgacauuaauuacuaaugaagaugaaaacuucgucaaagaugaucaacgugcugguguagaugcgaauuauuaugcuaaacaaacauaugauuacuacaaaaauacauuuggucgugagucuuacgauaaccaugguaguccaauagucucauuaacacauguaaaucauuaugguggacaagauaacagaaauaacgcugcauggauuggagacaaaaugauuuauggugauggcgauggccgcacguuuacaaauuuaucaggugcaaaugacguaguagcacaugaguuaacacauggcgugacacaagaaacggcgaauuuagaguauaaagaucaaucuggugcguuaaaugaaagcuuuucagauguuuuuggauacuuuguagaugaugaggauuucuugaugggugaagauguuuacacaccaggaaaagagggagaugcuuuacgaagcaugucaaacccagaacaauuuggucaaccaucucauaugaaagacuauguauacacugaaaaagauaacgguggugugcauacgaauucuggcauuccaaauaaagcagcuuauaacguaauucaagcaauagggaaaucuaaaucagaacaaauuuacuaccgagcauuaacggaauacuuaacaaguaauucaaacuucaaagauuguaaagaugcauuauaccaagcggcuaaagauuuauaugacgagcaaacagcugaacaaguauaugaagcauggaacgaaguuggcgucgaguaa

SEQ ID NO: 43 - RNA, 1548 nt, Staphylococcus aureus
augaaaaagaaauuagguauguuacuucuuguaccagccguaacuuuaucauuagccgcaugugggaaugaugauggaaaagauaaagauggcaagguaacaauuaaaacgacaguuuauccauugcaaucauuugcagagcaaauugguggaaaacacgugaagguaucaucaaucuauccagcagggacagauuuacauagcuaugaaccaacacaaaaagauauauuaagugcaagcaagucagacuuguuuauguauacaggggauaauuuagauccgguugcuaagaaaguugcaucuacuauuaaagauaaagauaaaaaacugucuuuagaagauaaauuagauaaagcaaagcuuuuaacugaucaacacgaacauggugaagagcaugaacaugagggacaugaucaugggaaagaagaacaucaucaucauggcggauaugauccacacguaugguuagauccuaaaauuaaccaaacuuucgcuaaagaaauuaaagaugaauuagugaagaaagauccaaaacauaaagaugacuaugagaaaaacuacaaaaaauuaaacgacgaucuuaagaaaauugauaacgauaugaagcaaguuacuaaagauaagcaagguaaugcaguauucauuucacaugaaucaauuggauacuuagcugaucguuaugguuuuguucaaaaagguauucaaaacaugaaugcugaagauccaucacaaaaagaauugacuaaaauuguuaaagaaauuagagauagcaaugcuaaauauauucuuuacgaagauaauguugcgaauaaagugacugaaacaauucguaaagaaacagaugcgaagccuuuaaaauucuacaacauggagucuuuaaauaaagaacaacagaaaaaagauaauauuaccuaucaaucauuaaugaaaucgaauauugaaaauaucgguaaagcuuuagacagugguguuaaagugaaagacgacaaagcugaaaguaaacacgacaaagcaauuucugauggguauuuuaaagaugagcaaguuaaagaccgugaauuaagcgauuaugcuggugaauggcaaucuguuuacccuuacuuaaaagacgguacgcuugaugaagugauggaacauaaagcugaaaaugauccgaagaaaucugcuaaagauuuaaaagcuuauuaugacaaaggauauaaaacugauauuacuaacauugauauaaaaggaaaugaaauuacauuuacuaaagaugguacgaaacacacugguaaauaugaauacaaugguaagaaaacauugaaauauccuaaagguaaccguggcgugagauuuauguuuaaauuggucgaugguaaugauaaagacuuaccgaaauucauccaauuuagcgaucacaacauugcaccuaaaaaggcagaacacuuccauaucuuuauggguaaugauaaugacgcguuauuaaaagaaauggauaacuggccaacauauuauccuucaaaauuaaauaaagaccaaaucaaagaagaaauguuagcgcauuaa

SEQ ID NO: 44 - RNA, 1695 nt, Staphylococcus aureus
augguguuauauaucauuuuggcaauaauugugauuauauugauugcuguagguguauuauucuauuuacguucaaauaaaagacaaauaauagaaaaagcaaucgaacguaaaaaugaaauugaaacguuaccuuuugaucaaaaccuugcacaauuaucuaaguugaauuuaaaaggugaaacaaaaacgaaauacgaugcaaugaaaaaggacaacguagaaaguacaaauaaguaucuagcuccuguggaagaaaaaauccauaaugcugaggcuuuauuagauaaauuuaguuucaacgcaucucaaugugaaauugaugaugcaaaugaguugauggauaguuacgaacaaagcuaucagcaacaauuagaagauguaaaugaaauuauugcguuauacaaagauaaugaugaauuauaugacaaauguaagguugauuaucgugaaaugaaacgugauguuuuagcaaaucgucaucaauuuggugaggcagcaagucuucuugaaacugaaauugaaaaauucgagccaagguuagagcaauaugaaguacuaaaagcugaugguaauuauguacaagcgcacaaccauauagcugccuugaaugaacaaaugaaacagcuaagaucuuauauggaagaaauaccagaauuaauuagagaaacucaaaaagaauuaccuggucaauuccaagauuuaaaauaugguugccgugaucuuaaaguugaaggguaugaucuggaucacguaaaaguagacaguacauuacaaagcuuaaaaacagagcuuaguuucguugaaccauuaauuagucgcuuagaauuagaagaagcuaaugauaaacuagcuaauaucaaugauaaguuagaugacauguaugauuuaauugaacaugaaguuaaagcuaaaaaugaugucgaagaaacaaaagauaucauuacggauaacuuauucaaagcaaaagacaugaauuauacauugcaaacagaaauugaauauguacgugaaaacuacuauauaaaugaaucugaugcucagaguguucgucaauuugaaaaugaaauucaaaguuuaauuucuguauaugaugauauuuuaaaagaaaugucuaaaucugcuguacgauauagcgagguucaggauaauuuacaauauuuagaagaucaugucacaguuauuaaugacaaacaagaaaagcuacaaaaucaucugauucaauugcgugaagaugaagcagaagcagaagacaaucuguuacgaguacaaucgaagaaagaagaaguguaucgucgauuacuugcuucuaacuuaacaagcguuccugaaagguuuaucaucaugaaaaaugaaauugaucaugaaguucgugauguuaacgaacaauuuagugaacguccaauacacguuaaacaguuaaaagauaaagugucuaaaauugugauucaaaugaauacauuugaagaugaagcaaaugauguucuuguuaaugcuguuuaugcagagaaauuaauucaauauggaaauagauaucguaaggacuauagcaauguugauaagagcuuaaaugaagcugaacgauuauuuaaaaauaaucgcuauaagcgugcgauugaaauugcagagcaagcucuugaaaguguugagccaggugucacuaaacauauugaagaagaaguuauuaagcaauag

SEQ ID NO: 45 - RNA, 1860 nt, Staphylococcus aureus
augccuaaaaauaaaauuuuaauuuauuugcuaucaacuacgcucguauuaccuacuuuaguuucaccuaccgcuuaugcugacacaccucaaaaagauacuacagcuaagacaacaucucaugauuccaaaaaaucuacugaugaugaaacuucuaaggauacuacaaguaaagauauugauaaagcagacaacaauaauacuaguaaccaagacaauaacgacaaaaaaguuaaaacuauagacgacagcacuucagacucuaacaauaucauugauuuuauuuauaagaauuuaccacaaaccaauauaaaccaauugcuaaccaaaaauaaauacgaugauaauuacucauuaacaacuuuaauccaaaacuuauucaauuuaaauucggauauuucugauuacgaacaaccucguaauggugaaaagucaacaaaugauucgaauaaaaacagugauaauagcaucaaaaaugauacggauacgcaaucaucuaaacaagauaaagcagacaaucaaaaagcaccuaaaucaaacaauacaaaaccaaguacaucuaauaagcaaccaaauucgccaaagccaacacaaccaaaucaaucaaauagucaaccagcaagugacgauaaaguaaaucaaaaaucuucaucgaaagauaaucaaucaaugucagauucggcuuuagauucuauuuuggaucaauacagugaagaugcaaagaaaacacaaaaagauuacgcaucucaaucuaaaaaagacaaaaaugaaaaaucuaauacaaagaauccacaguuaccaacacaagaugaauugaaacauaaaucuaaaccugcucaaucauucaauaacgauguuaaucaaaaggauacacgugcaacaucacuauucgaaacagauccuaguauaucuaacaaugaugauaguggacaauuuaacguuguugacucaaaagauacacgucaauuugucaaaucaauugcuaaagaugcacaccgcauuggucaagauaacgauauuuaugcgucugucaugauugcccaagcaaucuuagaaucugacucaggucguagugcuuuagcuaagucaccaaaccauaauuuauucgguaucaaaggugcuuuugaagggaauucuguuccuuuuaacacauuagaagcugaugguaaucaauuguauaguauuaaugcuggauuccgaaaauauccaagcacgaaagaaucacuaaaagauuacucugaccuuauuaaaaaugguauugauggcaaucgaacaauuuauaaaccaacauggaaaucggaagccgauucuuauaaagaugcaacaucacacuuaucuaaaacauaugcuacagauccaaacuaugcuaagaaauuaaacaguauuauuaaacacuaucaauuaacucaguuugacgaugaacguaugccagauuuagauaaauaugaacguucuaucaaggauuaugaugauucaucagaugaauucaaaccuuuccgcgagguaucugauaauaugccauauccacauggccaauguacuugguacguauauaaccguaugaaacaauuugguacaucuaucucaggugauuuaggugaugcacauaauuggaauaaucgagcucaauaccgugauuaucaaguaagucauacaccaaaacgucaugcugcuguuguauuugaggcuggacaauuuggugcagaucaacauuacggucauguagcauuuguugaaaaaguuaacagugaugguucuaucguuauuucagaauccaauguuaaaggauuagguaucauuucucauagaacuaucaaugcagcugccgcugaagaauuaucauauauuacagguaaauaa

SEQ ID NO: 46 - RNA, 2046 nt, Staphylococcus aureus
augaugaaaagucaaaauaaguauaguauucguaaauuuaguguaggugcaucuuccauuuuaauagcuacauuacuauuuuuaagugguggacaagcacaagcagcugagaagcaagugaauaugggaaauucacaggaggauacaguuacagcacaaucuauuggggaucaacaaacuagggaaaaugcuaauuaucaacgugaaaacgguguugacgaacagcaacauacugaaaauuuaacuaagaacuugcauaaugauaaaacaauaucagaagaaaaucaucguaaaacagaugauuugaauaaagaucaacuaaaggaugauaaaaaaucaucgcuuaauaauaaaaauauucaacgugauacaacaaaaaauaacaaugcuaauccuagggauguaaaucaaggguuagaacaggcuauuaaugauggcaaacaaaguaaaguggcgucacagcaacagucaaaagaggcagauaauagucaagacuuaaacgcuaauaacaaucuaccuucacaaagucgaacaaagguaucaccaucauuaaauaagucagaucaaacaagucaacgagaaauuguuaaugagacagaaauagagaaaguacaaccgcaacaaaagaaucaagcgaaugauaaaauuacugaccacaauuuuaacaaugaacaagaagugaaaccucaaaaagacgaaaaaacacuaucaguuucagauuuaaaaaacaaucaaaaaucaccaguugaaccaacaaaggacaaugacaagaaaaauggauuaaauuuauuaaaaaguagugcaguagcaacguuaccaaacaaagggacaaaggaacuuacugcaaaagcgaaaggugaucaaacgaauaaaguugccaaacaagggcaguauaaaaaucaagauccuauaguuuuagugcaugguuucaauggguuuacagaugauauuaauccuucaguguuagcucauuauuggggcgguaauaaaaugaacauucgccaagauuuagaagaaaaugguuacaaagcuuaugaagcaaguauaagugcuuuuggaaguaacuaugaccgcgcaguugaacuuuauuauuauaucaaaggcggucguguagauuauggugcagcacaugcagcaaaauauggacaugaacguuauggaaaaacauacgaaggaauuuacaaagacuggaaaccaggacagaagguacaccuuguuggacauaguauggguggucaaacgauacgucaacuagaagaauuacugcguaaugguagucgugaagaaauagaguaucaaaagaaacauaguggcgaaauuucuccacuauucaaagguaauaaugacaauaugauuucaucaauuacuacuuuaggaacgccacauaauggaacgcaugcuucagauuuagcugguaaugaagcuuuagugagacaaauuguauuugauaucgguaaaauguuugguaauaaaaauucaagaguagacuucggguuggcucaauggggucuaaaacagaagccaaaugaaucauauauugauuaugucaaacgcguuaaacaaucuaauuuauggaaaucaaaagauaauggauuuuacgaucugacgcgugagggugcaacagauuuaaaucguaaaacgucguugaacccuaacauuguguauaaaacauacacuggugaagcaacgcacaaagcauuaaauagcgauagacaaaaagcagacuuaaauauguuuuucccauuugugauuacugguaacuuaaucgguaaagcuacugaaaaagaauggcgagaaaacgaugguuuaguauccguuauuucuucucaacauccauuuaaucaagcuuauacaaaugcgacggauaaaauucaaaaaggcauuuggcaaguaacgccuacaaaacaugauugggaucauguugauuuugucggacaagauaguucugauacagugcgcacaagagaagaauuacaagauuuuuggcaucauuuagcagacgauuuagugaaaacugaaaaggugacugauacuaagcaagcauaa

SEQ ID NO: 47 - RNA, 2421 nt, Staphylococcus aureus
augacaaauaaaaugaagaaauggcaaaaauuauccaccauuacguuauuaaugaccggagugauugcuuuaaauaauggugaauuuagaaauguugauaaacaucaaaucgcuguggcugauacgaauguucaaacgccagauuaugaaaaauugaagaagacguggcucgacguuaacuacgguuaugaucaguaugaugagaauaaucaagauaugaagaagaaguuugaugcuaaagaaaaagaagccaagaaguuacuugaugacaugaaaacugauacgaauagaacauauuuguggucaggagcugaaaaccuugaaacuaauucuucucacaugacaaaaaccuaucguaauaucgagaaaaucgcagaaucaaugcaacauaagaauacgguauuaaaaacaguugaaaacaaguugaaaauaaaagaagcccuagauuggaugcacaaaaauguuuauggcaagaauccuucucaaaaagucgaggauuuaacuaaaaaucguaaggggcaaacuacacccaagaauaacucauugaauuggugggauuaugaaauugguacgccaagagcauuaacaaauacacuacuucuaauggaugauaugcucacuaaagaugaaaugaaaaauuauucaaaaccuauuaguacauaugcaccauccagugacaaaauuuuaucuucuguuggugaaucagaagaugcuaaagguggaaauuuaguggacauuucuaaaguaaaacuuuuagaaaguguuauugaagaagauguagauauguugaaaaagucuauagauucuuuuaauaaaguguucacuuauguucaagauucugccacugguaaaggucgcaauggauucuauaaagauggcucuuacauugaucaucaagaugucccuuacacuggugcuuaugguguuguacuauuagaggguauuucucaaaugaugccgaugauaaaagaaucuccuuuuaaaacuacacaagauaaugcuacauuaagcaauuggauugacgaaggguuuaugccauuaaucuauaaaggugaaaugauggauuuaucacgagguagagcuaucagucgugaaaaugaaacgagucauacagcgucagcgacuguaaugaaaucauuguugagauugaaugauaccauggaugauucaacaaaaacuagauauaagcaaaucguuaaaacuucuguuaauucugauucaaguuacaaccaaaauaauuauuuaaauucauauucagacauagcuaaaaugaaaaaguuaaugaaugauaguacuauuucuaaaaacgauuuaacacagcaacuuaaaauauauaaugacauggaucgugucaccuaucacaauaaagaccuggacuuugcauuugguuuaaguaugacaucgaaaaacaucgcacgauacgaaaauaucaacggagagaacuuaaaagguuggcacaccggugcaggcaugucuuauuuauauaacagcgaugucaaacacuaucgcgauaacuucugggcaacagccgauaugacuugucuuccaggcacuacuacuuuaaaugauaugccaucuacuaauacuaagaaugauaaaucuuuuguuggcgggacaaaauuaaauaauaaauacgcaagcaucgguauggauuuugaaaaucaggacaaaacuuuaacugccaaaaaaucauauuucauauuaaacgauaaaauugucuucuuaggaacuggcauuaaaaguacugauucaucaaagaauccaguuacaaguguugaaaaucgcaaagcaaauggguauaaauuauuuaaagaugauauugaaauuaccacuucagauguuaaugcucaggaaacccauucagucuuuuuagaguccaacgauacuaaaaagaacauugguuaucauuucuuagacaagccaaaaauaacuguaaaaaaagaaagucauacugguaaguggagugaaauuaauaaaagucaaaaaaaagaugacaaaaaagaugaguauuaugaaguaacucaaacacauaauacaucugacaguaaauaugcauauguuuuguauccugguuuaucaaaaagugauuuuaaaucgaagaauaauaauguaaguauuguuaaacaagaugaagauuuucaugugauaaaagauaaugauggcguauuugcugggguuaauuauagugauaauacuaaaucuuuugauauaaacggaauuacuguugaauuaaaagaaaaaggcauguuuguaauuaaaaagaaagaugauaaagcauauaaauguagcuucuauaauccugaaacuacaaauaccgcuucaaauauagaaucaaaaauuuuuauuaaagguuacaccauaacuaauaaaagugucauaaacucuaaugaugcugguguaaacuuugaauuaacuaaauaa

SEQ ID NO: 48 - RNA, 2427 nt, Staphylococcus aureus
augacauauagaaugaagaaauggcaaaaauuguccaccauuacguuauuaauggcuggugugauuacuuugaaugguggugaauucagaaguauugauaaacaucaaaucgcuguggcugauacgaauguucaaacgacagauuaugaaaaguugaggaacauauggcuggacguuaacuaugguuaugauaaguaugaugagaauaauccagauaugaagaagaaguuugaggcuacggagaaugaggcagagaaauuacucaaggaaaugaaaacugaaagugauaggaaauacuugugggaaagcucaaaagauuuagauacgaagucugcggauaugacucguaccuaucguaauauugagaaaaucucagaagcgaugaaacauaaaaauacuaaauuaaaaacagaugaaaacaagacaaaaguaaaagaugcacuugaguggcugcauaaaaaugcauauggaaaagaaccagauaaaaaaguugcugauuugaccucaaacuuuaaaaauaaaacuucuagaaauaccaacuuaaauuggugggauuaugaaauuggaacaccuagagcauuaacaaauacgcuuauacucuuacaagaagauuucacugaugaagaaaagaaaaaauauacagcuccuauuaaaacuuucgccccagauagugacaaaauauuaucuucuguaggaaaaucugaaccugcuaaaggcggaaauuuaguagacauuucuaaaguaaaacuuuuagaaaguauuaucgaagaagacaaagauaugaugaaaaagucuauagauucauuuaauacagucuucacuuacgcgcaaaauucugccacuggaaaagaacguaauggauucuauaaagauggcucuuacauugaucaucaagacgucccauacacuggugcuuauggcguuguacuauuagaggguauuucucaaaugaugccgaugauaaaagaaacaccuuuuaaugauaguaaccaaaaugauacaaccuuaaaaucauggauugacgacggauuuaugccacucauuuauaaaggugaaaugauggauuuaucaagagguagagcuaucagucgugaaaaugaaacgagucacucagcaucugcaacaguaaugaaaucauuguugagauugagugauaccauggauaagucuacaaaagcuaaauauaaaaagauugucaagacuucaguagagucagauucaaguuauaaacaaaccgauuauuuaagcucuuauucggauauaagcaaaaugaagucuuuaauggaagacagcacuauuucuacuaacgguuuaacacaacaacuuaaaauauauaaugacauggaucgugucaccuaucacaauaaaggcuuagacuuugcauuugguuuaaguaugacgucgaaaaacgucgcacguuacgaaaguaucaacggagagaacuuaaaagguuggcacacuggugcuggaaugucuuauuuauacaauagcgaugugaaacacuaccgugauaacuucugggcgacagcugauaugaaacguuuagcagguacuacaacuuuagauaaugaagaaccuaaaaguacggauguuaaaaagucuaguaaaacuuuuguaggaggaacaaaauucgaugaccaacaugcuaguaucggaauggauuuugaaaaucaggacaaaacuuuaacugccaaaaaaucauauuucauauuaaacgauaaaauugucuucuuaggaacuggcauuaaaaguacugauucaucaaagaauccaguuacaacgauugaaaaucgcaaagcgaaugauuauaaauuauauaaagaugauacgcaaacaaccaauuccgauaaucaggaaaccaauucccucuuuuuagagucaacgaauagcacucaaaacaauauagguuaucauuuuuuaaacgaaucgaaaauaacuguaaaaaaagaaagucauacugguaaguggagugauauaaauaaaagccaaaaggauauacaaaaaacugaugaguauuaugaaguaacucaaaagcauucuaauacagauaguaaauaugcauauguguuguauccaggcuuaucuaaagaugucuuuaaauccaaagcaagcaaaguaacugucguuaagcaagaagaugacuuccacguugugaaagauaaugaaucgguuugggcugguaucaauuauagugauagcgcuaaaacuuuugaaauuaauaacacuaaagucgaaguuaaagccaaaggaauguuuauucuuacaaagaaagaugauaacacuuaugaauguagcuucuauaaucccgaaucuacaaauuccguuucagauauugaaucuaaaauuucaaugacuggauacucuauuauaaacaaaaauacgucgacuucuaaugaauccggcguacgcuuugaauuaacuaaauaa

SEQ ID NO: 49 - protein, 412 aa, Staphylococcus aureus
IDSKNKPANSDIKFEVTQKSDAVKALKELPKSENVKNIYQDYAVTDVKTDKKGFTHYTLQPSVDGVHAPDKEVKVHADKSGKVVLINGDTDAKKVKPTNKVTLSKDDAADKAFKAVKIDKNKAKNLKDKVIKENKVEIDGDSNKYVYNVELITVTPEISHWKVKIDAQTGEILEKMNLVKEAAETGKGKGVLGDTKDININSIDGGFSLEDLTHQGKLSAFSFNDQTGQATLITNEDENFVKDEQRAGVDANYYAKQTYDYYKDTFGRESYDNQGSPIVSLTHVNNYGGQDNRNNAAWIGDKMIYGDGDGRTFTSLSGANDVVAHELTHGVTQETANLEYKDQSGALNESFSDVFGYFVDDEDFLMGEDVYTPGKEGDALRSMSNPEQFGQPAHMKDYVFTEKDNGGVHTNS

SEQ ID NO: 50 - DNA, 1239 bp, Staphylococcus aureus
attgattcaaaaaataaaccagctaattctgatattaaatttgaggtgactcaaaagagtgatgcggtcaaagcattaaaagaattgcctaaatccgaaaatgtaaaaaatatttatcaagattacgctgttactgatgtaaaaactgataaaaaaggatttacgcattatacattgcaaccgagtgttgatggtgttcatgcacctgacaaagaagtgaaagtacacgcagacaaatcaggaaaagtcgttttaatcaatggggatactgatgcgaagaaagtaaagccaacgaataaagtgacattaagtaaagatgacgcagccgacaaagcatttaaagcagttaagattgataagaataaagcgaaaaatcttaaagataaagtcattaaagaaaacaaagttgaaatcgatggtgacagtaataaatacgtttataatgttgagttaattacagtgacaccagaaatttcacattggaaagttaaaattgatgctcaaactggcgaaattttagaaaaaatgaacttagttaaagaagctgcagaaactggtaaaggaaaaggtgtacttggcgatacaaaagatatcaatatcaatagtattgacggtggatttagcctagaagatttaacgcatcaaggtaaattatcagcatttagctttaatgatcaaacaggtcaagcaacattgattactaatgaagatgaaaacttcgtaaaagatgagcaacgtgctggcgtagatgcaaattattacgctaaacaaacatatgattattacaaagacacatttggtcgtgaatcatatgacaaccaaggtagtccaattgtttcattaacgcatgttaataactacggtggtcaagataacagaaataatgccgcatggatcggtgacaaaatgatctatggtgatggtgatggtcgcacattcacaagtttatcgggtgcaaatgacgtagtagcacacgaattaacacacggtgtgacacaagagacagcgaacttagaatataaggaccagtcaggcgctctaaatgaaagcttttcagatgtttttggatactttgtagatgacgaggatttcttaatgggtgaagatgtctacacacctggaaaagagggagacgctttacgcagcatgtcaaacccagaacaatttggtcaaccagctcatatgaaagactatgtattcactgaaaaagataatggtggcgtacatacgaattcttaa

SEQ ID NO: 51 - RNA, 1239 nt, Staphylococcus aureus
auugauucaaaaaauaaaccagcuaauucugauauuaaauuugaggugacucaaaagagugaugcggucaaagcauuaaaagaauugccuaaauccgaaaauguaaaaaauauuuaucaagauuacgcuguuacugauguaaaaacugauaaaaaaggauuuacgcauuauacauugcaaccgaguguugaugguguucaugcaccugacaaagaagugaaaguacacgcagacaaaucaggaaaagucguuuuaaucaauggggauacugaugcgaagaaaguaaagccaacgaauaaagugacauuaaguaaagaugacgcagccgacaaagcauuuaaagcaguuaagauugauaagaauaaagcgaaaaaucuuaaagauaaagucauuaaagaaaacaaaguugaaaucgauggugacaguaauaaauacguuuauaauguugaguuaauuacagugacaccagaaauuucacauuggaaaguuaaaauugaugcucaaacuggcgaaauuuuagaaaaaaugaacuuaguuaaagaagcugcagaaacugguaaaggaaaagguguacuuggcgauacaaaagauaucaauaucaauaguauugacgguggauuuagccuagaagauuuaacgcaucaagguaaauuaucagcauuuagcuuuaaugaucaaacaggucaagcaacauugauuacuaaugaagaugaaaacuucguaaaagaugagcaacgugcuggcguagaugcaaauuauuacgcuaaacaaacauaugauuauuacaaagacacauuuggucgugaaucauaugacaaccaagguaguccaauuguuucauuaacgcauguuaauaacuacgguggucaagauaacagaaauaaugccgcauggaucggugacaaaaugaucuauggugauggugauggucgcacauucacaaguuuaucgggugcaaaugacguaguagcacacgaauuaacacacggugugacacaagagacagcgaacuuagaauauaaggaccagucaggcgcucuaaaugaaagcuuuucagauguuuuuggauacuuuguagaugacgaggauuucuuaaugggugaagaugucuacacaccuggaaaagagggagacgcuuuacgcagcaugucaaacccagaacaauuuggucaaccagcucauaugaaagacuauguauucacugaaaaagauaaugguggcguacauacgaauucuuaa